European Patent Specification EP 3 668 891 B1, published July 26, 2023. Title: New Uses of Proteins. Applicant: LGV-1. The sequence listing filed with the application follows.

SEQUENCE LISTING (2 sequences)

SEQ ID NO: 1 - protein, 575 aa, Homo sapiens
MLQQSDALHSALREVPLGVGDIPYNDFHVRGPPPVYTNGKKLDGIYQYGHIETNDNTAQLGGKYRYGEILESEGSIRDLRNSGYRSAENAYGGHRGLGRYRAAPVGRLHRRELQPGEIPPGVATGAVGPGGLLGTGGMLAADGILAGQGGLLGGGGLLGDGGLLGGGGVLGVLGEGGILSTVQGITGLRIVELTLPRVSVRLLPGVGVYLSLYTRVAINGKSLIGFLDVAVEVNITAKVRLTMDRTGYPRLVIERCDTLLGGIKVKLLRGLLPNLVDNLVTRVLADVLPDLLCPIVDVVLGLVNDQLGLVDSLIPLGILGSVQYTFSSLPLVTGEFLELDLNTLVGEAGGGLIDYPLGWPAVSPKPMPELPPMGDNTKSQLAMSANFLGSVLTLLQKQHALDLDITNGMFEELPPLTTATLGALIPKVFQQYPESCPLIIRIQVLNPPSVMLQKDKALVKVLATAEVMVSQPKDLETTICLIDVDTEFLASFSTEGDKLMIDAKLEKTSLNLRTSNVGNFDIGLMEVLVEKIFDLAFMPAMNAVLGSGVPLPKILNIDFSNADIDVLEDLLVLSA

SEQ ID NO: 2 - DNA, 1728 bp, Homo sapiens
atgctgcagcaaagtgatgctctccactcggccctgagagaggtgcccttgggtgttggtgatattccctacaatgacttccatgtccgaggaccccccccagtatataccaacggcaaaaaacttgatggtatttaccagtatggtcacattgagaccaacgacaacactgctcagctggggggcaaataccgatatggtgagatccttgagtccgagggaagcatcagggacctccgaaacagtggctatcgcagtgccgagaatgcatatggaggccacaggggcctcgggcgatacagggcagcacctgtgggcaggcttcaccggcgagagctgcagcctggagaaatcccacctggagttgccactggggcggtgggcccaggtggtttgctgggcactggaggcatgctggcagctgatggcatcctcgcaggccaaggtggcctgctcggcggaggtggtctccttggtgatggaggacttcttggaggagggggtgtcctgggcgtgctcggcgagggtggcatcctcagcactgtgcaaggcatcacggggctgcgtatcgtggagctgaccctccctcgggtgtccgtgcggctcctgcccggcgtgggtgtctacctgagcttgtacacccgtgtggccatcaacgggaagagtcttattggcttcctggacgtcgcagtagaagtgaacatcacagccaaggtccggctgaccatggaccgcacgggttatcctcggctggtcattgagcgatgtgacaccctcctagggggcatcaaagtcaagctgctgcgagggcttctccccaatctcgtggacaatttagtgacccgagtcctggccgacgtcctccctgacttgctctgccccatcgtggatgtggtgctgggtcttgtcaatgaccagctgggcctcgtggattctctgattcctctggggatattgggaagtgtccagtacaccttctccagcctcccgcttgtgaccggggaattcctggagctggacctcaacacgctggttggggaggctggaggaggactcatcgactacccattggggtggccagctgtgtctcccaagccgatgccagagctgcctcccatgggtgacaacaccaagtcccagctggccatgtctgccaacttcctgggctcagtgctgactctactgcagaagcagcatgctctagacctggatatcaccaatggcatgtttgaagagcttcctccacttaccacagccacactgggagccctgatccccaaggtgttccagcagtaccccgagtcctgcccacttatcatcaggatccaggtgctgaacccaccatctgtgatgctgcagaaggacaaagcgctggtgaaggtgttggccactgccgaggtcatggtctcccagcccaaagacctggagactaccatctgcctcattgacgtggacacagaattcttggcctcattttccacagaaggagataagctcatgattgatgccaagctggagaagaccagcctcaacctcagaacctcaaacgtgggcaactttgatattggcctcatggaggtgctggtggagaagatttttgacctggcattcatgcccgcaatgaacgctgtgctgggttctggcgtccctctccccaaaatcctcaacatcgactttagcaatgcagacattgacgtgttggaggaccttttggtgctgagcgcatga